European Patent Specification EP 3 488 242 B1, published June 11, 2025. Title: THERAPEUTIC AGENTS FOR NEUROLOGICAL AND PSYCHIATRIC DISORDERS. Applicant: VIB VZW KATHOLIEKE UNIVERSITEIT LEUVEN, K.U.LEUVEN R&D. The sequence listing filed with the application follows.

SEQUENCE LISTING (18 sequences)

SEQ ID NO: 1 - protein, 33 aa, Homo sapiens
NVDSADAEEDDSDVWWGGADTDYADGSEDKVVE

SEQ ID NO: 2 - protein, 17 aa, Homo sapiens
DDSDVWWGGADTDYADG

SEQ ID NO: 3 - protein, 9 aa, Homo sapiens
DDSDVWWGG

SEQ ID NO: 4 - protein, 10 aa, Homo sapiens
GGADTDYADG

SEQ ID NO: 5 - protein, 72 aa, Homo sapiens
TSEGCQIIHPPWEGGIRYRGLTRDQVKAINFLPVDYEIEYVCRGEREVVGPKVRKCLANGSWTDMDTPSRCV

SEQ ID NO: 6 - protein, 657 aa, Mus musculus
MLPSLALLLLAAWTVRALEVPTDGNAGLLAEPQIAMFCGKLNMHMNVQNGKWESDPSGTKTCIGTKEGILQYCQEVYPELQITNVVEANQPVTIQNWCKRGRKQCKTHTHIVIPYRCLVGEFVSDALLVPDKCKFLHQERMDVCETHLHWHTVAKETCSEKSTNLHDYGMLLPCGIDKFRGVEFVCCPLAEESDSVDSADAEEDDSDVWWGGADTDYADGGEDKVVEVAEEEEVADVEEEEADDDEDVEDGDEVEEEAEEPYEEATERTTSTATTTTTTTESVEEVVRVPTTAASTPDAVDKYLETPGDENEHAHFQKAKERLEAKHRERMSQVMREWEEAERQAKNLPKADKKAVIQHFQEKVESLEQEAANERQQLVETHMARVEAMLNDRRRLALENYITALQAVPPRPHHVFNMLKKYVRAEQKDRQHTLKHFEHVRMVDPKKAAQIRSQVMTHLRVIYERMNQSLSLLYNVPAVAEEIQDEVDELLQKEQNYSDDVLANMISEPRISYGNDALMPSLTETKTTVELLPVNGEFSLDDLQPWHPFGVDSVPANTENEVEPVDARPAADRGLTTRPGSGLTNIKTEEISEVKMDAEFGHDSGFEVRHQKLVFFAEDVGSNKGAIIGLMVGGVVIATVIVITLVMLKKKQYTSIH

SEQ ID NO: 7 - protein, 616 aa, Mus musculus
MGPTSPAARGQGRRWRPPLPLLLPLSLLLLRAQLAVGNLAVGSPSAAEAPGSAQVAGLCGRLTLHRDLRTGRWEPDPQRSRRCLLDPQRVLEYCRQMYPELHIARVEQAAQAIPMERWCGGTRSGRCAHPHHEVVPFHCLPGEFVSEALLVPEGCRFLHQERMDQCESSTRRHQEAQEACSSQGLILHGSGMLLPCGSDRFRGVEYVCCPPPATPNPSGMAAGDPSTRSWPLGGRAEGGEDEEEVESFPQPVDDYFVEPPQAEEEEEEEEERAPPPSSHTPVMVSRVTPTPRPTDGVDVYFGMPGEIGEHEGFLRAKMDLEERRMRQINEVMREWAMADSQSKNLPKADRQALNEHFQSILQTLEEQVSGERQRLVETHATRVIALINDQRRAALEGFLAALQGDPPQAERVLMALRRYLRAEQKEQRHTLRHYQHVAAVDPEKAQQMRFQVQTHLQVIEERMNQSLGLLDQNPHLAQELRPQIQELLLAEHLGPSELDASVPGSSSEDKGSLQPPESKDDPPVTLPKGSTDQESSSSGREKLTPLEQYEQKVNASAPRGFPFHSSDIQRDELAPSGTGVSREALSGLLIMGAGGGSLIVLSLLLLRKKKPYGTIS

SEQ ID NO: 8 - protein, 669 aa, Mus musculus
MAATGTAAAAATGKLLVLLLLGLTAPAAALAGYIEALAANAGTGFAVAEPQIAMFCGKLNMHVNIQTGKWEPDPTGTKSCLGTKEEVLQYCQEIYPELQITNVMEANQPVNIDSWCRRDKRQCKSHIVIPFKCLVGEFVSDVLLVPDNCQFFHQERMEVCEKHQRWHTLVKEACLTEGLTLYSYGMLLPCGVDQFHGTEYVCCPQTKTVDSDSTMSKEEEEEEEDEEDEEEDYDLDKSEFPTEADLEDFTEAAADEEEEDEEEGEEVVEDRDYYYDPFKGDDYNEENPTEPSSEGTISDKEIVHDVKVPPTPLPTNDVDVYFETSADDNEHARFQKAKEQLEIRHRNRMDRVKKEWEEAELQAKNLPKTERQTLIQHFQAMVKALEKEAASEKQQLVETHLARVEAMLNDRRRIALENYLAALQSDPPRPHRILQALRRYVRAENKDRLHTIRHYQHVLAVDPEKAAQMKSQVMTHLHVIEERRNQSLSLLYKVPYVAQEIQEEIDELLQEQRADMDQFTSSISENPVDVRVSSEESEEIPPFHPLHPFPSLSENEDTQPELYHPMKKGSGMAEQDGGLIGAEEKVINSKNKMDENMVIDETLDVKEMIFNAERVGGLEEEPESVGPLREDFSLSSNALIGLLVIAVAIATVIVISLVMLRKRQYGTIS

SEQ ID NO: 9 - protein, 36 aa, Homo sapiens
EESDNVDSADAEEDDSDVWWGGADTDYADGSEDKVV

SEQ ID NO: 10 - protein, 24 aa, Homo sapiens
GTPDPSGTAVGDPSTRSWPPGSRV

SEQ ID NO: 11 - protein, 32 aa, Homo sapiens
KIIGSVSKEEEEEDEEEEEEEDEEEDYDVYKS

SEQ ID NO: 12 - protein, 36 aa, Sus scrofa
EESDNIDSADAEEDDSDVWWGGADTDYADGSEDKVV

SEQ ID NO: 13 - protein, 36 aa, Gallus gallus
EESDNLDSADAEDDDSDVWWGGADADYADGSDDKVV

SEQ ID NO: 14 - protein, 36 aa, Rattus norvegicus
EESDSIDSADAEEDDSDVWWGGADTDYADGGEDKVV

SEQ ID NO: 15 - protein, 36 aa, Mus musculus
EESDSVDSADAEEDDSDVWWGGADTDYADGGEDKVV

SEQ ID NO: 16 - protein, 35 aa, Xenopus laevis
EESESFDSADAEDDSDAWWGGADADYVDRSDDKAV

SEQ ID NO: 17 - protein, 35 aa, Danio rerio
AGKESESAAVEEDDSDVWWGGAEADYTENSMTRDA

SEQ ID NO: 18 - protein, 35 aa, Danio rerio
EQKDLDSEEQEEANSDVWWGGAETEYTDASVLKEQ